European Patent Specification EP 4 161 942 B1, published August 2, 2023. Title: Improved oligonucleotide synthesis. Applicant: Bachem Holding AG. The sequence listing filed with the application follows.

SEQUENCE LISTING (2 sequences)

SEQ ID NO: 1 - DNA, 10 bp, Artificial Sequence
  thymine-rich test sequence
ttttattttt

SEQ ID NO: 2 - DNA, 20 bp, Artificial Sequence
  test sequence containing all DNA nucleotides
ataccgattaagcgaagttt